European Patent Application EP 4 130 280 A2, published February 8, 2023. Title: TARGETED INTEGRATION SITES IN CHINESE HAMSTER OVARY CELL GENOME. Applicant: Development Center for Biotechnology. Application EP 22171570.9, filed December 19, 2017. The sequence listing filed with the application follows.

SEQUENCE LISTING (18 sequences)

SEQ ID NO: 1 - DNA, 6192 bp, Cricetulus griseus
  gene 1..6192: note = Srxn1
  misc_feature 3900..3928: note = n is a, c, g, or t
  misc_feature 4660..4672: note = n is a, c, g, or t
  source 1..6192: mol_type = genomic DNA
agcttgaaaatcagtcccaagagtatttatttccagcagagtaatggcagatgctgtaagctaggggcttcccccaaacactaggtgcggagtatttatctacatccatgtgaacaatataccctgtgctcacttagtacacacttgggagacacagtacacccaggaggcaaggacagtctcaccctgacagggtttctgtcccaggaacagactgaaggaggaagtgaatcagggagtgataaacactatgaagacagtcttacagatgacaagccaggatggaaggaggccatgggtctgtctgaagtgacaggggcacagaaccactagggaggctacggaagctacaaatatggactagtttaggttaagagcccaaatgcctaagccatggctcctctgaagaacagtagggaccagtactgggcaggtagcccctatgttcaacgagcagggcagtgggtgaagtccgggaggactccttggaagggtggccctggacagctgcatttggtaggccttgtgttgaaggtgtgagagggtaggtttaagaatgctcccactggggctggagagatggctcagaggttaaaagcacagactgctcttccacaagtcctgagttcaattcccagcaaccacgtgatggctcacaaccatctgtaatgagatctggcaccctcttctggcctgcagacagaatattgtatacacaataaataaacaagtaaataaataaaggcccctctggatgcccatttcctaatctttaggacctgtgaaacccaccttacatagtggaaatctgctgatgggagtgggctttaaggctcctgaaactgatagattgtcctggattacccaggcaggctgaatgtaatcaccaggttctttgaaagcaaaaggctgtggcaaaagaggtcaccagctgctgctattttgaagataagggagaggccctcagcttaaagggttcaattgttaacttgatgaaatccagaaccactttggagggtgggcctttatggatgcctgtgggggtttatagtggttactttaactgagatgggaagaaccacccactgaaggtggcatcattctctaggctgggatcctgtactgtataaagagaagacactgagcagtgcacaagtggtttttcaccattctgactggcgatacactgtgaccagtggcctcaagcccctgccatcatgacttccctgatgtgatggacggtatccttgaactgtgagccaatgtaaaccttgttacccttaagttgcatttgtcagggcgatttgtcccaacaaagggaaaagtaactgagacttcaggaaatgcattttcccttaaggcctcaagaaaacagtcctgctggctccttattttagctcaataaaacacactttgagctgggtctggtggggggtacctgtaatcccagcaccagagagatggaaggtttcagactagcaaggctatatagagacacaccctgctttaaaagcagcaaaacaacaacaacaacaaacaacaacaacaaaaaaaaaacccacaaaaaacacagctttggactcctatcttgttttaagccatgtttgtgacaacgtgtttaggtggccaaagcagataggtccttgtctccacaagagcctgtggctccagcatgggacagaggtttctaaactggtcttttaaacccatcaggatcccagctgtgctagggggcacccaggtggctgtgaggtcacagaaggcctagcccaatagggtgggcaggggagacattgacaccaagacagaaagactaagcagttagaagcaacaaagagataaaaactcgggcttcagggcattggtgatgctcccgctgaccgtgccagagctcctaagtgcaatccctagcatcatgtgcacaccaaaactaaaacaatgccgagaaggaggtgtgggagcacttcctggggtgaggtaagtctatgcaaaggcccagtggtactcagagagcggtggggctaagtccccttcccacagtcagcttgaaggcaactgccaaggtggcaaaataattgcttttgtgaaattctcacaggaagacaggggtgcaaattttaagaccaaacatcctcgggactttaggggttccagggcccactgctcaagaatctggaagaatcttgatctgacacaaacgccctagcttctgcggggactctccctccaatatggaggccttgagcctctcctacttcccaacatacatgacacacccagaccactgccctgactgtcatggccagaagagacatcaggatacccaggttatctgggggtaaagtttcattgtatcatcttgtaagtgcttgacctaaggcaagttgcttaaaaaacagaacaaaacaaaacaaaatccaagcttcctgtgcctcagtttctcctccatacaggaggaaccgcagctacttcacagagctgatcagagaagctgaaatcagctgggagcaaccgcagcacttttgagtatgtgcgtcacagatcattactttcatggtcaagtccaagtgaggaacctgaggcccagggaggctccgccagcccagcccgtcaaggtcacacaggcgaagctgagctcccgcagatcctggacccctaccctcgcgccctctctttctcgcgcgggccggtaggctccgcgggctcaccaggatcgtgtccacgaggctctgcaccttggccgggtccagcacggatggcagaggccggatgagcacgctgattggcacgttgtgcaccgtggtgatgcagcccgagtggatgctgcctcccttttatttccagcagagtaatggcagatgctgtaagctaggggctttcaacccatctaccgactgccggctgcggcgccccgccaccccctcgcgacacacgcagtggacgcgtccgccgctgactcagggtgagtctgcaagtcgcggagcaaagtcgcgagtgacgcacagagcggtgactcaggctctgagaggcgaggacgcgggaggtcagacctgcccagcaagaaagggttggctctcagtgggagctgggaacagtggcccccacatggggaaaacaggaatgtggtgacctcacacttcagagccaccctgctagctgggcacaatgttaatcccattttacagaggaggaaactgaggcacagagaagttacgtcacacacatacacacccaacacacccacacacaggcttggagctaatgagtgggtgagctgaggcccaaaccccggcaggctcgctccacggatctctctagattccaccgcgggctcccctgggctcagcgacaagaactagccaccgcgccttctggagttgtgttgattctgtacgtccttccatgaaattccatattgcacatccccaagctatatccaggaagtaggagtgggagtggttactgaagggcctccccaaagtagtccccctgcggggtgggggtggggagagaggaaaagaaaccaaagtcaggttacccgactgcgcagctagagtccggctggagctgtggcggggtgtcaacccgaacagctgcacacgccctttcctgtggcttgcactgcctcctagctggcgcgtgatgtccagcgatgagcgtccctagaaaggctgggcctattccaggtcagcctggacgccgtacaggacccactctgtgactttctattgggaagctgatacaagccttcccaggcccaagggaaggggacagtgaaagagcctgcggtttgggacctctgggaccgctcttaggagagagagctgcggatggaggtgacccggctaggtgctagagaaaggaaccgccaaggcagactcggctaacggggaggggctnnnnnnnnnnnnnnnnnnnnnnnnnnnnnaggactctgcatcactctagggacagagactctgccccctgctctttcctgggcaagtgtggctggaggtgctgagcctagccttacctggctaccctgcttttgagcggagcaggcatcttaggggcccagaagcacacagcggtctgcctagggtgacccgaggtaatcaaaggatcacaaagctggctggctggagtaggaggtgtgaaggaaagttcccagaaaaacaaacgacgacaacaacaacaacaacaaagcaaaacaaacaaacaaaaaaccatcttcaccgaacattacaggctgatggacttacaaaacttagtgattgtggagaggttggaatgttgccagtccagagccaaatatcctacactatccttaatcgtccccgtaactgtttattgcccgccctcgtgtgacctaacttccttttaggatacactgatacacaactagctgacacaaacccacaagttcaggatgtctcccctggcatcacaggtacagacctgtctctgatgtcatagctcacttccccggatgtatatggttttaagccattgattaattcatgttggtgtctgcagagtccagaagagggcatcagatcactagggactggagttaacagaagaatgtgagcctcttgtagatgcaggaattgaacctgggtcctctggaggagcagccagtgctcttaactgctgagccatctctccagcccctccnnnnnnnnnnnnngattttttttttttttttttttttaagatttattatgtatacagctttttgcctgcatgtattccagcacaccagaagagggcactagatttcatcatagatggctgtaaaccaccaatggttgctgggaattgaacccaggacctctggaagagcagccagtgctcttaacctctgagctatctctccagccccccacccccaccccaccccctggatgtattttaagtgtgttgatttacctactttctttgttctatttctgctaataattcataaaactgttatcatgttggaacgtggacttttaggtgacctaaatactccagagtacactcttacccctgggagacgacgagagctgtgttttttatgttgccataggctcttgctccccgattccttctgcttcccccacctcagctgatggacttggaggtgacacagacagagaatcctgtttatgaaacatttggacatacaggtgactttccccaagtgtttggaaggtgaaaggattatgggtccttccgtttgaagcccctccccaacctgcttgaccatttctctagcttaggcgtcagggctggctttccatgttgtttgtcccacagcacctcattctttggtgttcactgagcatttctttgggggtgcagaggcagctttgcactccatcttctcacagtctcaagagagctgccagtgtgaagccggtctcacttttgttcacacccaggagagggagggagggagggagagactacaccagcagtggtgacatcaagtgctttctttagtcagtctgattgggctagcttgagtcacccaggatgactggcattctccagggatatgccgtgtactgagccgttaaagcatggagtctgtcaccaagggggacgactgtgatgaatttagaggggacagtcaaccacccttctgggatacagcctcttctgagtcacctgtatgtgggtgaaataggtgggccgatcctgggtgaatatgaggctagtgggtgagagatggatgctgacaagagaaagatgcgccagaggcctgggtgtcactgccttgtcctttagccccctctgatgttagctgcaattgtgccagaaagttctacagcagatgactcactcagcaccaccagcccttaacccaggtgccctgagctcccacgttgatctctgcccacacacagcacatgccagtgctgtcatatttgccgtgggagtagaacacgccagtcttccaccaacacaggttggcaatattaatcatttggatctttctggactgttctcagagatcagtggtaaccagcctgttgctctagcaggggcttcacagacacacccctgacattcttcctgctgctcactctgccacttgggctcccacttagcttgcacaagggcctggagcctctgcctttgtcagtgggaaactagaacctcagctaagagcaccatacattgccataccctataatttatgccccacctggcttaaaa

SEQ ID NO: 2 - DNA, 192 bp, Cricetulus griseus
  gene 1..192: note = Srxn1
  source 1..192: mol_type = genomic DNA
cacagagcggtgactcaggctctgagaggcgaggacgcgggaggtcagacctgcccagcaagaaagggttggctctcagtgggagctgggaacagtggcccccacatggggaaaacaggaatgtggtgacctcacacttcagagccaccctgctagctgggcacaatgttaatcccattttacagaggagga

SEQ ID NO: 3 - DNA, 6164 bp, Cricetulus griseus
  gene 1..6164: note = Adh5
  source 1..6164: mol_type = genomic DNA
acctctaagactgtggaaccccattctgatctctattacagtggctgggagacaagctaactgggtaactggaaaaacttgggggctaagactatgatttaatggttataatgaaggagtcttatttaccatacaacaattcatagtccctttacatgggcccatcccagttggctcaaatccagttatgaactccttggttcaactcacaggaccaccccttcccaggacaatcatcccccttaataatgtcagtcccactagaaaactctcccagccccaaggaccaataaatcatgcttttctctcctactggctatagatgtttactataaataattataaataattctcagtcaaactggaccagacctgttggttatgtttagacccctctcctccctactatgagggcataacagtcatttcttcatacaaagaaaattcttcccgcataacctgcccatagggaacccaccccaagcttacattaggatcagcccactggcctttgtatcctgccatctaacaaacccattctggaggcttatctgcccctctgagattccacctacttattacagcacttgcaccgcctgttacctcacagcacctgaaggcacctagtgggcatgctccatgtgtacacacccagatactacaacaaaactcagaattctgtgtcttcattcagattttcccccaagtcctttattattttgatgagaccatgacaacccacctagccaccttccctccacttgacaaaggtagtctccggcactccacgttccaactttggcaggtctgggaatagttggggttacccgaataggcactactgcccttgtgttacaatatgaaaattacaagacgttaggtgccttgagtgatcaagatccggccaagttagaaaaaaatctatttcccacctagaatcatcccttagttctttagcatcctcagtgctacagcaccacccaggattagacctcctcttccaacagggaaaacatgcctggagctgggagcacaatatcgcttctaatcactcaggggtgataaaagaatctgtgcctggtatgtaaaaggttacaatatcgagaaaaacaatggaggaacagttctgattggcacgaacccttgttctcatggtcatcatgggccacgaccttaataaccgcactggtaggacccctattgatcctgttgctagttctgatttggagcgatgtatagtcaacactctcctccttattataaaagaattcactggagcaattaaatgaatggtcctttgcagccaatataggcctctgcctacaaatgacacagaactcacattaagttcaaacatttgacttttgttttaactcaaggggggaatgaaggaactagggccagttgttttttaaggggccagtttgctaagacctctgccccatattaccccataatcctatgactcatgtcggacttcaatcagaccctcaggaagtatgccgggcccggtggccaatcgggtcctacctgaccacacgtaggaactgttcttgctatcttcaaacagaatcttggcacagcagactgaaccctgacacagccaccacagctgctgaccagatgtcattggccaatcactaaagtctctcctgaccagtcagggtctccacccaaatcacttcatgcctaaccacagctggaattgccctaagcaagcttaaaagggaccacctcactcctccctgtagttggtgccactttgggtggaccccagcatgcgaatttttctgtcttgagaacaaagctgctttctgcaattgcatgtctgtggtcttctggtcattaggggcgacctaagggccctacactgtgattctcgggtttctggctggagcaagtagatggacacacctgccatcaacacggagatgtaaagaaaggtccctttaagaagaaaatacaagactggttttaagtgagttgagttttaagcactatgagctaccctaacacacacgggtatctagcaggcactttgcacttcaagcctggagtttaggaaagccaccctgactggagacagaatccggtagtcaccctataatcattttataagttaaaagtcggagtgtgagttagtgtgaaaagagggaaggacttcaaagagttttgtggaaaacgtcaacccttaaggtcttgtgttgaagaaataagccttggaaaatacaaagagaatgcggtgtctttgcaggcacatttcaacaaaacctccgtgtgtcctggcagcgtttaggattacgtaagaacgcagcatcctccggctatacacagacgctctactctgaaaacgcacccattctgtccctcgttccgtgtcctatggccccgggaagctgctggacccggagccagggcaggtgcttctaggacggcccctctcgccccagagtcccgcgttaccacgactcgccgctgggggcagtgttgacgcatcccgtacccggaagcgccaagcggggggagggggaggcacggaaggcggggctagttcctcacgtgcttcaggggcactgggtttcctcgcgttgttcctctctcacgtctaagccttacgtgcgagggctcaccaaagttaggcagggaaataccacagagacgctttgcagcgactccgtcagaccagccccgaataaaaagcgtcaccgactctggataaaatccccgccctcgccagcaggggagcgcgggagccaaaacccaggctccgcccttccggcgttagccccgcctccctctcaagctccgtccctctgcacgcggcctgagcatcaaggtcccgcctcccgcgctcggccccgcccctcgcgcacggcccgcccattcccgggatccgctaggcttgttgcggacgttttgctcgcgaaccacagcttgcggacatggcgaaccaggtattgaaacgcggcatgggcccgagcggaggaagggagcgcccgtggggtatgccgccgccagcgggggaggcgacggcagggaggctttgtttcggccctgcgcttgggagcagcccgcgggaagaggcgggatggagtagcttgcccggatcgcacttgcaggatggcgatggcgtagctgagcactggccgcgctcaaaactgccaagcaaagtcaggctcttccttgggccttcgctttccgtgtgcaccaccgtgtacatgtttctttaaatcacgtcttaagtgtttattgactttcaagcccatctcctgtaaacccggtggcttgcaacctttattctgtcgacatatttcgtaagcatcaagtgaactaacaaaacccaacattcctcattaggttcgcttctggggtaaggaagagctagctcattgctttagatgcacgataaaaaaactgtatatggagttttaaactttccaagaaccacatttgagaaagaatagataaaagtaattctaatgctatgtttacccaacttaatagtcacagtattgtttcaaattgttagctgggatatttttactcttctaagctttcaaaatttacatccatagccaatctcgggtcaccctgacttttttctactgttcagtagccacacatggcaaatggttaatgcattagctagcacagttactgtggggaaaaggggccagccaaagaaacgcaccctgagcagaaccacagaaacacactttggccctagaatcagccaaatttgactcgaaacctggcagaaaaccatccaatccctgagcacaagatctagccagtctgagcttagtgattgaaatctgaccaatccccaccctataaatctccctgggaaaactccacccctaagaatccttatataaaccctgtacctgttcagcttctgactgcttgagctgccagctgtcctctgccaccctggaattagagccaggtgaggtttgggtgagaccttccttcaccactggaatggagcaagcaaggggagcagggctgtaacacttttgctggggaaaccttcccctagcaaagtgaagttgttaaactctggggaccagagcctaactataacaatttcacctgggaagccctcccctgctggagcagagctgttacactagggaagtcttccccctggagcagggctgtaagctactacacttgttgtgacttgtggtattccttggctcccgattgccagaatacttttccacccgagctgtaacactcagtatcctgtggctcccgagtgccaaaattccatccaatccaccacaatgcttaaagctacgagagatggttatggtatttttacatatcccccatttggatttttttaggatcctttccactatgtagttttgcactacagtggtgttttgtaagctttaccaagggaccccaggaaactagtggctttcagcagagagcaggtacatagggacccttcaattacttaccaaacctactgacaggacctgggtgggattttgttgtttctcttacctggcttgtcttttgctgtgttggggatcgaatccagggccttgtgcattagaggcaagtgctctgccactaagctaagcaacatccctagctttttggacaatgtctcactatatgactcttgctggtccagaactttatgtgggcctcaaacagagatcctcctgcctctgcctcccaagtgctgagattaaaaatgtgtacctccacacccagcaggacctgtatctaatctgttcttttccatacattgtacagtgtcatgagcatttcaattagatcttttttttaaaatagtgtttactgtgtgtgtgtgtgtgtgtgtgtgtgtgtgtgtgtgtgtgtgtgtgtgtaccacgtgcatgcagaagcttgtggaagatacaagaaggcatgggtcctctggaactggagttacaagtagtcttgggcatgtagatactgagcactgaactgagatactgagtcctctgcagagtgacatctcttcagcctttcgaatagtgtgtgggggcgggggttgtagtagtggtttctccagggagggtttgagataggctctctctatgtagccctgtcctgcaacttgaaatgtagaccaggctggcctcaaactcacagagatccacctgcctctcaagtactggaactgaaggtttgcgtcactatccctgaccctccaaatatatgtttttagtatatgaattatatgaaacctaaaaaacagttctccatttcacacagaggtatacgtttttctgtgaatgtgctgttcactttagttgtgtgtgtctgagtttgtaatgtgtgtgagagtgtgtttgtgtatggtcacgtggaggtctgaggctgacatcaggtgtcttcttcaatcactctgcaccatctgtattgaatcagggtctttcacttgaacccagagctcaacagtacagttagtctagccagccagcttgctctgaggacccccgtctgcagtctgagtctgccatctgtaattacagacaggccgctacatcaggtgtgctgtggagttgcgctctggtcctcatgctggcacagcagggcctctacccactgagccgtctccccagccctggtacacgctgacattagcatcatcgttatctgaactgaccatgaaatagttattaatttaggaggataaactgttcacttccttccccccactctaggtgatcagatgcaaggctgcagtcgcctgggaggccggaaagcctctctccatagaggaagtagaagtggcccctccaaaggctcatgaagttcgaattaaggtaatgtcacagcaaggcactgtgggaagaagcttacagttaggtcttcggagagaagagtggacctgagggccacagaggattaacccaaagggttgagtcgaggagaaagcactggaagccttccaactgcagagtcacagagccctctcacctgccccccccccttcattctgtattgctctggggctgagaagaagccaagcccccggattagtgtactatcacgacataactttttatggtttgggtttacggtggctttatatgatcctctcccttctgctgatcccataactcacagtgtggtggattagagtcagtaagaatagacacaagcttcag

SEQ ID NO: 4 - DNA, 163 bp, Cricetulus griseus
  gene 1..163: note = Adh5
  source 1..163: mol_type = genomic DNA
ggggtatgccgccgccagcgggggaggcgacggcagggaggctttgtttcggccctgcgcttgggagcagcccgcgggaagaggcgggatggagtagcttgcccggatcgcacttgcaggatggcgatggcgtagctgagcactggccgcgctcaaaactgcc

SEQ ID NO: 5 - DNA, 6429 bp, Cricetulus griseus
  gene 1..6429: note = ASPDH/JOSD2
  source 1..6429: mol_type = genomic DNA
gagtgacacagcatgaggccccagaggcccttggatactgcttccctccccagaacagccactcaccacccactgacctgtcaccctctacctgtcaagtccagctttggttttgtttaggcagggtctcaggtgtcccagatatgcaccactacagcagttcatggggtgctggggatggaaccccagcctcatatacatgctgggtaagcgttctgccaatggagccccagcccctcaacgttttgttatttgcctttttgagtcagggtctctatatgcaacccaggccagcttccaattcagttttgcctcaggtcaacaggctggtctcactactcttaaccccatttcctcagtcatgagtcactcatgtcacttggaccccccacagaatacctttcactggtaccaagtttatcagtttagctcatcagtcagtcagtcagtcagtcagtcagtcagtcagtcagtccccattagccagaggctctctggcaaaaacctcccccatctaccttcaagtcaccctctgcttcatcccacaaacccagggccagtgtagcccacagcctaggccctacctcctcctgtcccaccacacagcggccaggcccaggccttgcagggcagccatgatcacgttgacatcataattgccggtgcccaggaggctgcgatgagggttcagccgggagtctggggccagcctgggggtgaagggggcagagccaaggttgggaatcctggaaaggccttcaacttctcacacagcaggagaggcccagagcctggcttttggctctttctctttaagccccacacagctcattgggctctaagccctgtttttcctcccattcccaacacctgtactctctgcctagctaaagtttttgtctttttccactcagaaacccttcccagtctctagtctctccatccgatccacctccaaaagccttgagctgcctgcctctctcctactcccacctctcccatgactcccaagtgctctggacaaagtctctgcccttccatctgcccttctcatcatggcctctttccagaccagcctcagatgtcatttcttctggtagagaagccatcaaacccccagaatgggcacagagctcccctgagtgacaatgccgctcatgtcaccatatttgaatacagaatgcctctttcatttggcaataccctgccctactctgttcacagccctccctggtgccccaaatcccggggacagactctcacctcctccagtggcaagtggttcttgcatagcctcagcaccagctcttaccagccacctatctccagctgtccctgtgcccaagccttccctctaagctctctccagatgtgaccctgttcctctgaagagctggccccttggagagcagtgacatggagggaaccacttgtgtttgctctgtgtcccgagccttctcctcactacatctgccttagctctagttgttcagcatgctcctggcatgacagagctggtggcagggggatggatatctcctaacataaatctacagtctgagggtgctggctgagcagcagtgagaagatgtgaaggctgcctctggatgtggacatgaactgcaggctggggtgttggcgtatctgtgaaaggattgtggggcctagaagtgggactaggaagagagtttaagaaagtgatggttgaaattctgaagggcacctacgtgaccaagaagaacaagaatgcctgggtaagagctcagaatcaccacagtggggtcatctggggccaaggagagtagtgaaggagaagctgcagactggtaggcaaggaccagagcacccaaagccttggagttcaggctgaaggacctgggctattctctaggagtgccagggacccccagaggaataaatgcagaggagggggaaggcagctgtggggctgtgtgtaggatggtcaggaggagaaacacagacagctgggaggctgtgacaaaggctcagataagagaggttgaggccaaagctgggttgaggctgtgagaagcagcaggtggaagggcagacatcagctccaggatctgcgccccggccttgttagtgcccaggcaggctcccatgcccctcagccctgctcttccagggccaggacctagggcagtcacctcttgcaaatttcatctgcagcttcctggctaaagagctgttgttggaggacgttgttgagagcgtggaccgcgcacagctctagccgctgccgctcgtggtacactgagggtgggctcggccgcgcttccggggcctgagacatgccctcctcggctcctgctgggggtggtacaaggagaaagtgttagggacccaggatctcggccatctgggtctccagactcctgtgtccctgggcaacagccactgagatgggcactggagccagcttgggaggaaacgacccagctacctaggctgtctccgaagcgtagaggcatctttatgccctagtcctagggggaaagggctcttttttgctcacttggcaatagagatccacccccacttcatgtctctaagcaaaaaaaagtccggatcactataacctagtaacgaagtatcgccccttctgtccctaggaaacaatacctttttggttcccaagcaacagagtactccccacccgcttggtaaccggtccgatttctgatcacctagcaatggaggactcctccttccccgtctctgggtaacagggtctcttctggtcgcctagcaacgaaagacttcccctcatcaataaccagggttctctcctcccgtcacctggcaacaaggccctctcccagtcactaagcaacaggagctcccctcttcctgtcacctggcaaccaggcacgctcccacccgcctccgcacggcactcgcttggccctcaccccgtcggcctctctgctcgctgggaccggccgctttctcattccctgggtagcggccgagtggtaccacgctgactgggcaggcaggacggactacagctcccgaccgcccgagcactcctgactgcaattcccgaaggcctccgaggcgcctaaataggacgcgcggtacggaagtccgccggggacgctctgcagcgcggaactacaactcccgtcggaccacacagccagttttcatgcacccccagggctcactgcagtctagaggtttctgggaaatgtagtaactggggctctcgcgatagcttccaggaaaatggtttgtgcgtatgctcgtgcgctcgctgctatggcgtcacacacagtgtgttgaagcgtgatgtaatagagttaggggataaggaactaaagaggccaaagagaacagccgacagaactctgatgtttactgagacacacagtggtcgaggtgacagcaagggcagcgggggagacttgtcagcagaggtgaatcccaggtctggaggggagctggcagcagcctgtggggagaatgaaagactagaatgaccacacagacatgcaagcagccatggcggccgtgggctttgaaaatgatagtgtagtacaacccaaagaggatactcagaaagagatgtggggtgtggatgcagagacaagaggggggctgagactcagagaaaaagagagacctgggagagaaaactaaggatgggcaaagacagacaaccggggtgggacatccgacatgtgagttctgcagggcacaaaagtcaagggactcttggagaggtctggacgcacccagtaggctgccccagaaggctgtgacagtagcagagccggtgacagcgccaggctgggctgggttctctctgtgggtgtgcacagcaaagctgtggcctgtgggccctggggggcctttcagctccacgtccaccacgtgcatgtctttgaggctgcagccagcggagaagggtagttagtacatctggcctgtacacaggtgggccacttacttccgttgctcacctaaggtcagccacaagcaccccaatgacacggtcgaagcctagactgggggcagccagggcagcagctgccatggtgttagaatttcggggggccaaggggcagagcccacgcacagggccctcgtagagcactgtgcgcggcccactgatgtgtgctgcagccagggacccctccagtcggaagccatcaggatgtgtggccatggtgactcgaaggctctggaaacaatggcagggtcaggaagctgagactcttacatgttccctcagttgcagcccatatggttctcacctggaggcctcccgatgcatccaatctcctgatgtcttcagtcccccacagggctcctcgggccacaaacacagtgtggccccagcagtttgatgcctccatgagctgctgctctgtggtctggtcagccagagctgagggagaccccaccttgggaagtatggtagagagagggaaggccaagacatagatcattgctgtgtggtgggatgcagccaacacagagaagggcttgctgagggattagggggctcaccaggaggttagcatgtcgcaggatttgtacccctgattcatggattatatttggatgggccacttctaccacaaggtcaggatgcctgggagagggagacatggagtaggcccttagagaagaatcaggtctcagggtttggagggatgtcactccttaccctggctagggagggaaatgggatggtgggtgtattctagtttatctttatgtgcactgagacccagagagggtcaaagtgttgtctgacactgggaggcaggcagtaaggctcccactgtgctgtgggccactgacctttccttaagggtagtaaggtcttggagctgcagggcagggggcacactccctgccattcgtccagggtcacggttccatacaaaaacaagttctaggcccagttctggtccctgagccagaaggcgagacacaagagactgtcctgcagaaggggagagccagagatccaaggaaagtacagagactacaccccagtcatggagatggagagggggacagagagagatacacagacacagaggagggggagggccagtgacccaaggaaagtacagagaacacatcccagtcagagagacagaggagagagggacacacacacacacacacacacacacacacacacacacagagagagagagagagagagagagagagagagagagagagagagagagaaagactatatagacaccaaaaggggagagacagagactcagagacacacagaaagagggacaaagacctagaaagagaaaaagagagagagatgagaccaagaggaaagatagaagactgagatacctcagagacccagagagagaacagagacctagagagaggcagacacccagatacacacacacacacacacacacacacacacacacacacacacacacagagtgggggggcacgacagagaggaccagagagaggaaggcccagcaagtgggcagaaggcagactgagctggcagactggggagaaagacaagtgggagcagatatttctgggacattagggatagggccacaggaggaggccctaggctagtttggactcacccaggcggccatagcctaccacccccaccttctgggggacttgagggactacactggtggccatggcctttagcacggtgtcctgttgtagatcttcagtgtttgttggtctctgtaccagacctgggcagtgaatgatctttgtagtttaacccttgaccctctccactggagccagagggagggagcagggtggtagggatgaggtgcttctctgtgagccctctgccctcctgtgctggctggcatggtggcttgcgagctaggcctttgtggccctgtgtgctcactaccccactgcctcctgtgcagccacattctcccatccctcatgaggtgcagtcccccctcctcaggctgaacagcaggttgtcatggaaattgcattttgcttgggataggggaagaactggggactagaacttgggtcttccactaggtcccttacagacctcttgatctctgttatgtggaaaggtctggctggagtgtcatgtggttcggcatgccacactgtgtcctgtctttctcagtcctccatgcccctcagtcccggccagagtcccctcccccaccccagtgtctaattgcccttgaggtcacagtctcctgcctctttgtattcctggtcccctgcctcctctcccacctcctatcccagccacgaagaagggggtctgcatagctgggggagttcctaagtgtccccaggatgagtccagccactgcctgtcaggcctggcatgggacatggcaggctgcagtaggccagctccctgcccccattgccacctggtac

SEQ ID NO: 6 - DNA, 255 bp, Cricetulus griseus
  gene 1..255: note = ASPDH/JOSD2
  source 1..255: mol_type = genomic DNA
taccacgctgactgggcaggcaggacggactacagctcccgaccgcccgagcactcctgactgcaattcccgaaggcctccgaggcgcctaaataggacgcgcggtacggaagtccgccggggacgctctgcagcgcggaactacaactcccgtcggaccacacagccagttttcatgcacccccagggctcactgcagtctagaggtttctgggaaatgtagtaactggggctctcgcgatagcttccaggaaa

SEQ ID NO: 7 - DNA, 6538 bp, Cricetulus griseus
  gene 1..6538: note = Tenm3
  source 1..6538: mol_type = genomic DNA
cagttaccttgtgtacatcacttacaacgagcaattcgaagagaaagctaaaataatttcctggacaacaccatgaaacaggctaaaatacttaggaataaaccaagttataaatgtgaatgttttatatagtgggagtcagaacacaatgctgaatgacattaaagcaaaccctaataaatgacatcttgggttaacaaagtgacgttcagacacaaagcaatccccataaaaccttagcaatgtctgctacagctgcatgcgtttgaaacatccaaaaacgcttacaaaatacacaaagctggaggacttaggtaggcttatgtgaaaatatattagtaacctctaataactagtatggtactggcatagagaaaaataaatcaaagcaaacggttacgtaacaaagagtattattaaatgttcacatatatgatcttgacaaggtaccaaagctacaccgtgtgggggtgagggggacagtctcttgggcgaatgacgatgggagaactggatgaccaggcacgtttggggcttactgttcattacatacaaaaatcaactcagaaggaattaaggagatatacagagccctaacattctaaaattcctataagaaaacatgaaacattcctgacattatatttgacgatgacttcctggatgtgacaccaaaagcactgtcaacagacactaaatagggaaatgagtgaatcttgctagtttgcaaagcttctgcttaggtgggcttgggagtgtgtgggaggcgggcatagtgctcacctttgaattgcctaagggctaaatcccgcggccaaagctccgccctttttctccgagggtgggggccagtgacctcacgagagctcgtcctcaagtagaaagcaaagaggacaacttcccgccggctttggtggcgcaggccggtaggatttgctgaaggaggcagaggcaggaggatctggagttcgaggccagcctggactacacatttttttttcttccaagtaaatatccacaactacacggttcatgagattactcgcaggatttaggattttaaagaataatagtaaacagaagcaaggaagtgatcgggtttgaggaggtcacacctctttaatgcacttaaagaggacaggaatacagtcccagctgaagtccaagagaagacagacaaagggaagggcgcacttaatacagaggaataaatactgaagggagctcgggctgaaatggagctagaactgaaaaattcaatatcccatctgttagggtcacccgaggacaggacaccagacaccttcaggcaaacagcttttatatgtgagaggagtcatggagagaaccagaccagagcctagccagacagagacctgttccgtaccatagtctaacggctgctttaaacacagtgtgggcttaaatgtctttcatgtcaggaagggaggacggcttgggagcattgccaggccacacataacactttggtggagactaaacaggatggtggtctctttgtccttctttcaaggcctcctggaagatttactaaggaaaggggattactggggagatgtatcaaggtttttatacacgcaagggcattgctcggccctgtggctgcatctggttttcattgccctggctctcaagggagtctccctcacatagggtcaagcaggagataggatgtcaggaccgggagacacagcagagaaactggagaacaatatctttaaatcaaagaaagaaaaaatatttaaaaggaatatgcaagaatttggggacaccatgaggcccaaacttatgagttacccgagaagactctcaggtggaagaaaatgaatggggtatccagagaagacccatggttgcaatgcttgtcttagttgtgaaccacactccagcagtccacaatctcttgaccaactctcaaatgccatcatctgttgaatattcccaggaattggtccatgagttccctgaaatccctcaagatctgataatgctcaccagacccgtcctcacagacactcacgagatatgctccactaatttcccaggtatttcctaatcttagcacgttgacaatcaaggctgagcatcccaacagcataaagttgaccaaggagcacgggaaaagttgcacagcatcgctactcatcctgaggattaaagtgaaaacaccacgaggaaagattcctggtttgtcgctttgcttgaacgagcctggaagtttgcagctcatcctcacacagacaccctggtgaaccaactagaaacctagcagttctcctaggctgtgcaagaaaggtgagcacacacaggaggaaatacataaagagactggagttcagcgttgaagtcagtaggtcacaggcaccctgggtccttgtcacacttgcctgaccctgaccccgccggcacaagagggtctggttctgcggttcctttactcgcagcaattgagtctggttcccaagaagacgccccacgcaggacgaggagagcgagcgggttggaaggaatccacggccggaggtgcgggagtgtttcccggggtgaccagcagggggcgcggggcgggaaaggccttcggggctcctgaagttggggttcccgggaatgaggggagtgtgtgagccgggcgggctgagagcaggttagagccaggccgagagcggttggggagaaggcgaactgggcgtggtagttttcactctacactccgcccacagtgttgggagggcgagtacgtcatcgtaactcagcgctaactaacggtttgatgtgagctgcttccgccggctctggtggcgcaggccggaaggatttgctgaaggaggcagaggcagggggatctggagttcgaggccagccaggactacacatttttttttcttgtcctccaacaaaacatccacagctacaggctacagtaaaattcctacacccacaaaggctctccacactctactctcaacctcatttcgctcgcgactgacacccaaccgacaccatcttttctagacgcacaggcgcctgctccaccctgctgctcacaagcctttgctcacacaccgactcacacgctccacctccgcgctggccaatgctcgcatagtctaacggctacttgaaacccatagtgtggacttaaatgtcttttacgtcaggaagggtggacggcttgggagcattgccaggccacacataacactttggtggagactaaacaggatggtggtctctttgtccttctttcaaggcctcctggaagacttactaagcaaagcggggattgctggggagatgtatcaaggtttctatacacgcaagggcattgctcggccctgtggctgcatctggttttcattgccctggctctcaagggagtctccctctcattgagaagactcagtggaaagccttcctagttgacatagggtcaagtaaagacagaatgtcaggacctgcagacacagcagagcaactgggaaacaataccttaaaaacaaacaaagaaaaatatttaaaaggaatatgcaagaatttggggacactcatgaggcccaaatttatgagttacctgagaagactgtggggtggaagaaaatgaatgcggtatccagagaagacccatggttgcaaagcttgaccagctctcaaatgccatcatctgttgaatattcccaggaattggtccatgcgttccctgaaaaccctcaagatctgataatgctcaccagacccgtcctcacagacactcacgagatatgctccactaatttcccaggtatttcctaatcttagcacgttgacaatcaaggctgagcatcccaacagcacaaagttgaccaaggagcacgggaaaagttgcacagcatcgctactcatcatgaggattaaagtgaaaacaccacgaggaaagactcctggtttctagttttgcatgaaggagcctggaagtttgcagctcatcctcacacagacaccctggtgaacctactagaaacctgacagttctcataggctgtgcaagaaaggtgagcacacacaggaggaaatacatagagagactggagttcagcgttgaattgtcctccaacaaaacatccacagctacacactacactaaaattcctacacccacaaaggctctccgcactctactttcaacctcgtttcgctcgcgaccgacacccaaccgacaccatcttcttcagacataatgactgtcagtgtacaaattaaatgaattatttactaggagctgaaagaccattgcaactgctcgccaattcgactatttgagctgaagccggagttgtctgctccacatatttctttccatcaataatataggcggctctcccattggaggagccatcagtaaaaactaacatagcattttttacaggattgcttttaacaatttttggaaatataaaaggatgcattagtgtaaattgcaacagtccatgagctggaaactgaatatcaattctccctaaaaactgatcaaaagcaatcgcccatgaatcactgttttggaacaacccattaacctgatgcttggtgtaagggacatgtattatatttggctctttgccaaaatacttcctagcttttacaaggcatttttgtaccatgcaggctactgcttcaaaataagggtctaatactttggatggcgagactggtaggtgtagccagagtaatggtccctcctgccacagaacagaagtcggactatgccttgtggggagtatataagcctcccatggctttgcatagtcaatataacatatttgttgacgctgaatcgcctcctccaattgtagcaggactcgtctaccttcctctgttagctttctaggtgaatttggatcattatctccctttaaaatatcacagagcggtttcaaatcaccagtaggctctctttaaaaaggacgtaaccattgaatattccctattaatttttgaaagtcatttaaggaccgtaagctatcttttttaatctctaatttctgaggtctaatctctttagcatataacatatgacccaaatattgaaaaggtggctgtctctgtaccttctctggagcactcactaagcctgctctcttgagactttgctgtagctgtccataaatctcgagcagaaccgcttcatatttatggacaagtaaaatatcatctatataatgaacaataaagacttgtggaaatctgtccctaaccatttgtatagctcgagacacaaacttttggcataaagttgcactattggccatgccctggggtaaaaccttccaatggtacctcctcatggctctttaaaattaactgaaggaatgctaaatgcaaacctatgacagtcctgaggaaccaggggaatagtataaaaacaatcttttaggtctacaacaatcttataagtaccctttggtacagctgcaggaatgggtaatcctggctgtagtgctcccattggctgcatggttttattaactttcctcaaatcttgtatcagcctccatttccctgatttctttctaatcacaaaaataggagaattgcatggggaattcgaaggctcaatatgaccactgtccagctgttcctgcaccaaccgctgagcagcctgtagtttctcttctgttagaggccattgatctatccatattgactcatcacttttccatacgatgggatctgcatggcgtgcaggcttctcagtgacctcagctaaaagtgtcctaaccctgcattgggatgtctcctgctggctgaggcgggaacaacattcctctcactgccctggtcccctccttgatggggcgacaacccttgctgagatacccgattagcaacaattgcacttgggctatacaagtatattcccatccgggccataacatctcagccccacaaattcacaggcaaatgaggaagaatgaatggctgaaaagtccctttatgacctttagcatctctccaataaagctcatcgctactctgttcaggattcttcgtctgaccaattccttgtaactgagtaatagtctccattttcggccacgtggaaggccattgactggctgtaataactgacctatccgggcctgtgtctaaaaggccggaaaaagcccttccatttacatataatctctgggcgttgaggaccgatagcctgcaaccaataggcatcagaagaaccaaacccagaatctcctctcttaattctcttaacctgattgtttgtcctcacctggggaagcaaaatcaactgagcaagcctctgtcctgaactcatcaccgaaactccatcaggagaatgaatcacaacccttgtctctccttcaaaatcagcatcaatcactcctggaaacaaaaattccctgcatcgttgtgctactcctccctagcaacaatccaacagttccactcggcaaaggtccataaacaccagtgggtaacgctgatatctccatctctggcgttaaaactgcgtctgtggctgaacaga

SEQ ID NO: 8 - DNA, 538 bp, Cricetulus griseus
  gene 1..538: note = Tenm3
  source 1..538: mol_type = genomic DNA
cgactgacacccaaccgacaccatcttttctagacgcacaggcgcctgctccaccctgctgctcacaagcctttgctcacacaccgactcacacgctccacctccgcgctggccaatgctcgcatagtctaacggctacttgaaacccatagtgtggacttaaatgtcttttacgtcaggaagggtggacggcttgggagcattgccaggccacacataacactttggtggagactaaacaggatggtggtctctttgtccttctttcaaggcctcctggaagacttactaagcaaagcggggattgctggggagatgtatcaaggtttctatacacgcaagggcattgctcggccctgtggctgcatctggttttcattgccctggctctcaagggagtctccctctcattgagaagactcagtggaaagccttcctagttgacatagggtcaagtaaagacagaatgtcaggacctgcagacacagcagagcaactgggaaacaataccttaaaaacaaacaaagaaaaatattta

SEQ ID NO: 9 - DNA, 6200 bp, Cricetulus griseus
  gene 1..6200: note = SIVA1
  source 1..6200: mol_type = genomic DNA
atctttcccaatggtcatgtagggtcagaagcgcacaaggatcgcctaaagctcgtcttacctacaacttacattcagcaaagcaggagaagcccgtttcccagggtgtgaggaaaggcctttcacagagccagacaaaagtgggcgggctcatctagtgtacctgcctttaaaacaaaacgactgtatgtctgtggcctgcacttgacactggggtggcttagtgacactgtcctgctaagcttgggagagtgccagtgttacctggtgtgtgatatggatgtcaggaccaaggtgttataacagctggactcctacatttttggtgtcatggagctacagtgtggtgcttgttcaggaaaaagaaaaaaaaatgcagcaagtccttgaaagacagaccaggtatatcacatttcccagaactaacagtctaagaacgtacactccagagctgccagggatccaggaataacaattcttcctgtctccagggacagagcagcccagacacacacacttggtcgcagtccctggaaacttctccagactgaagcagacaggtcttaattagcatggcctgtgctcgctggaacaccaagtggccccttgagtaacatgccggagtctgggggtacattaggctagcccagtctaaggacatgtctcattgcattttcacctctatgacaaaataactatatttaaaaaaaaaactaaaaagggtttattttggatgactgtttcatccatggccagtcatggccagctcggtggctagagctctatgtgaggcagaagcatcatggtggagagcacttcatcaggaaggaattagagagacaggggaaccactcacccttcaagacgcacaaccaggtctcacctaaaagcccattcagccatgaactcaccgagggatggatgaatccattgaagttaggccatcatgatccaatcacccttcaatcatgctgccatctggggaatcacgccttcaacatgtggggcctctgaggagagacttcacattcataccacaccacccaggaaaggctcacactaaacctccctgagcccatcaggtgggttagagaggtccctgaggaccaagcaggaggaaaatcacaataacattcttgaataaaacaaccctattcctaaccctttggaaagctgccagtttgcttagaagataagcacatgtccccctctccctctaacacattcacgttcggagggaagagggagccccattcccgagtagcacccaacactgaatgatcaatatgtcagaaaaggcctggtccaaggttgtccataggaactaaatgcatcatagccaaagcttgccaatggccctggtgcctaacaggcagatacacaactttaggctttctagacagaagaacacccagtatcaaaacgaaccagctgccacagacttgaactagagggagcaagctcagaactacgggagagcagccagatacatcggcacacacagaatgagtactccctgtatgagattctgatgccatttggtgggaactttggaaaaagagtaagaaaaagctcagtgtcagacattttacaagcatactctggctgtggcccccaactgaagggaaaagacagaagaaactatgacatgattacccctctctaacacccaccggcagccagacccagtgaaaccctttggaagcttgcagggaattgtgggaattcttggccgggtgagggggtgggggtgtcattatcttaatgtgaacagcagtcctggtggtggttccctagccatgttcccgccccgtctgtcccactggatttaagccttacagtaggagacaagcccatgcctccacatagaggtggagcctgttccttacagttctacaacaggggacaccacccacggggaaggaaacacagaaggcagttgtcacttctacaggtgtttgtcatcagggctttaacctgtacacctacttggcacttgtcctatgctattcatgttgaagtcctaactcctaagacttcagaatgtgactatctggatacagccttttgtttattttatttttggtgttttgagacagggtcgcaccacacagcttgggctggcctcaaactcacagagatccgcctgcctctgcctccggagagctgggattaaaggcgtgcgccgccaccacacctggctcctgggtatatatatattcttaacgagttaaaacggggtccttagggtggacccgaactcaaagaggttggtgtttttatgagatgaggactcagacaccccatgtagtttccatctgcagatcaaggaagatgagaggcctgcagagaacccaacgccttaatctgaggctgtgcctttgtaattacagatcccctaattggccttctccctttccgaactcgggaacgcaaactcaagtactgggactgggggtgagggggtgtgtgtctcaaaatctggagaatgctgagcatgcgccaggcctccctcgcaccgtgatgagcgcaaaactcaatgcacctcaacaagtcgcccttaggttcagatagagtgtggaaagaatacaggactcaggaggccctcggcaccgctgctgtgccgactgtgtgcaccgcgttaggagccgcccaggcaggcagtgccagcggtaaacgctcacccaagctcgggctcacggacgcaggaggaccgcagggagagatgggtgccggcacccaccctgctgctgcgactcgtcccccgggaagaccacccatcacagttgctaagcgaccgcggagactttgtgccgcgcaggcttacacagagccccggcgcgtaagccccgcccctgggtagcctcccgctggtttcccgcgccacaccctccagagcccccgcctcttaatcctcggcctatcccgagtcgtctcgcgcactacccccgcccacctccaactctcggcctatcccgcgccgcgccacgcgaagaccccgccctccttgccatccctttggcctttcccgcgccccctgagttccacccacttcctccctcagcctattgcgcgcccttgagccccgcccccggcctctccccggcctatcgggctccgcgccgtcgccagccccgcccccgccggcgttgtgagcgcgctgtgacgtccgcgccgctgtggtcagtgtttggtacccgctgccatgccgaagcggagctgcccgttcggggacgcttccccgctgcagctcaaggtccatgtgggcccgagagagctgagccgcggggtgttcgcccagcgctactcgcgggaggtcttcggtgagtgcggagttccgtggtagggcgcgcagcgccgcgccgtgggagaccccaactggcttgcgcgtcgccatccccggggggggaggcggcgtggggggggtccccggggagcggctccgggggaaatgcgagtgtagccgaggactgtcgagcgggagtcggccccctcaagtgggctttctggcggcagggtgttgctttgcagtgatggctctctggggccgatgcaacgcggcttacctggcttagggcgaagtttatgcctgtagttttgagtggtgcgctgtgcctttgggatgtgtcgttaaagcccaggctgcggaattacagactccctaatgcgccgtgtgtgtgtgtgtgtgtgtgtgtgtgtgtgtgtgtgtgtgtagctgatgggccctttccctttctgtactgtggaatgcaaactcgagtgctgagacctcaggggtgatgagtgaagtgtgaggcctgaacagcaaagcgtcatgcactcatttaaaagaaacaaaagtagacatgacgggagtcttggcattcgcccttgatgctagcaactcaccaggcagaagcaggcggatctctgagagttccggggccagcctggtctacagagcgagtgccaggacagcctccaaagccacagagaaaccctgtcttgaaccacccccaccccccaaaaaaaagaaaacctaagtataattggaacctagcagcctggctctactcttttaaagacttatatcctggagcacttgccagggccagtcagaaccagccaggtcagggaggggtgctggtttctggggtgttgtatagtcatacagtacacacaatttgaggcctgaaggatgaataccaagcctcggcctacactctggactcttttgtgggccaggagtccttgaggagaaagattactctcaacatgggaatcttcctatctccctctttttcaagcaggcttttacaatgtatcttaggctaaccttgaacttaaacactcctgctgcctcagcctcctgagtgctgggatgtgcctctgtatctactttctatcttaaagcaggaggtggcacagactgtaactggcctgataacagccactccctgtgactttttgctggctgttgctgctgccagtttcacagaggggcccctgggtctgacaggtctcccctggctgtatgtgggagtgagcatttctggaaccagcacacagtgtagcctaatgggaagcccctgttaaagcccacttagcgctgggatagggggtgggtggacctggaaggttctgggagacctttgtcaggaggttgctgtctttgtcccctatagtaagtgcagttgtccgctggcctgatggtgattgtaggcgctgttttgaacctgtgtgtttcctgcctctttggggcacttgctctggagagtgagtggttcaaggccagagctttctctggcgtgaaagacaggtgcttataggagggtgaagagtaagacactaacccagtgaagtaaggttagctgtggctgctgagataggctaatggaaggaaccctgcgcccagcacatcggggtggtggggttgggctgcagcatctgcaggctgctgtggaaggagcgaacagtggagacagaaaggacgggagcattttcagcttggaggcagggaggccctggcagtgtcaccacttagggaacaggcacagaggacgacgcctatgcaggggctttgcagttggcagtgttgtctttaggaaggatctttcttccccagaaagaaccaagcagctccttttccaaggggcccaggcctgtagagaccacatatggggtgaaagatgtcccatcatccacctgccggagtcactgaagcctggcctggtgggggcccctcaagctgcaaggggacagatgctgattggacctgatggccgactgatacggtgcccagctcaggcctcagaagctggtgagtggctgccagcggtactcgctggttatcacacctaggaaacaccttggcaaatgctctcttcaggggctttgacaaccttggcaagtagcatccgcttagagcagtggttctcaactgggtcacgaccctttagccaatctgtctccaccacgacatgaactatattaaaggttgcagtgtcaggaaagttgagaaccactgactttgaacctggtaagttgagcaaatggcagaaggtttggaagcctcctgttgttgggaggtctgcccctcagagacatccaggagtggaagtcagcagcttccagttgttgtatcggaaaaggaacagggctctcctggtatcctgtctgtagtaggaacatgctggtccattgcctgtggaaaaatgagctcatgtgactggtgaaggcaggcctctgtgtcagcgctaaatctggctggtcccagaaacctcctggctgaccagcaaaacagggaaccatatcttgagacctagacagagacacagagttctgatagagtactccagggaagagtgacccttccatgctaggactaggtgggtgatatgccctgggaatgcctcgctgtggatctttagtgccccaggtggctgatagttataaggactcagtggctggggcaggtaggtgcccactgccctcgtgttcttccagtttctttccagtgccggtggtgttttttcctcacaggtctgcctgggacagctcccatcgcttgctcatcctgtgtgagatctgcagatgggaaggcggtctgcagccagtgcgaccgtgccctgtgtggacaatgtatatacacctgctggggctgcggtgccttggcctgcatgctgtgtggccttgcagagtgagtgctctgacctgtgggg

SEQ ID NO: 10 - DNA, 199 bp, Cricetulus griseus
  gene 1..199: note = SIVA1
  source 1..199: mol_type = genomic DNA
gccctccttgccatccctttggcctttcccgcgccccctgagttccacccacttcctccctcagcctattgcgcgcccttgagccccgcccccggcctctccccggcctatcgggctccgcgccgtcgccagccccgcccccgccggcgttgtgagcgcgctgtgacgtccgcgccgctgtggtcagtgtttggtaccc

SEQ ID NO: 11 - DNA, 6200 bp, Cricetulus griseus
  gene 1..6200: note = SYNE1
  misc_feature 4064..4073: note = n is a, c, g, or t
  source 1..6200: mol_type = genomic DNA
atgttggaaatactctttgagcaggtgggcctggtggtatggacctgtcatctcagccactggtgagcctgaggtagaaaaatctcatgatcaaggtctgctaggctacacaagtgagtgcaatgctagcccaggcaacttagtaagaccctgcttgataggaagagcaaaagcaaacaagggtgggagtggggaaaatagcagtgaactgcttcctttgcagcactgcaaaagtgaagaaggaaaagaaatacttcttgaaatgctaattctactagttagtatacaaaataagttgtggaactcaaaagcatttagtgtctttcttgtacagcattattaagaagagctcagtatttttggcagcgtaggaaaaaccaagtgacaaattacttgaagccagtgattattgtctattggcattgacacaagcagtttcatttaaatgacagcccaagagatcagttttactctaagtgcgttttaaagcttagagtggttctttagaaatcaacatttctcaataaaatcatcctgattttggggatggaatgttaaaactgtacataaatgcactcggtgctttggttttgggatccctttgtgttgaaataacacgaaaagttgggtggacaggggcaaggagtcctaactataccaggcactcaactctgagcagctctctcccccagaatcttatggtccagaggttggtcatgtgaaaagtatcccaggcttgtgccatcatctagagccggagtttgagagggttgtgagccatcatgtgggtgtccagaggtgaacctggggtgtctggaggtgaactcaaagattttctgcaagaccagccattgatctcagacttttctccagccccttttcctctcctgtttcttttagcaagtcttctatttcaggagaccttgacctgcagggatgcccaggacctgcacatttcaaggggccatttccttctcaggtcagagtggctctgttgccattaccattttcataaccatcccattttaaatttcctaggtctccttaagacgacagcaagtgagtgaacgactgaacgaatgggctgtcttcagcgaaaagaacaaggagctgtgcgagtggctgacgcagatggagggcaaagtctcccagaatggagacatcctcattgaagagatgatagaaaaactcaagaaggtgagctgtggagtgccttcgagagtatccaaactttagaggaggagctaaaatagacatataaaatctatcttcatttattttttaatttacttttggtgtttttttttttttttttgcatgtgcatgtttgtatagtgtgcatgcatgtgtgtatgtgcctcttcacatgtgtgtggcaccccggatgagcatgtgcttatggagaccagaggtcaaagttaggcatctttctcagttgcttttagtcttttaaattgatgtggggtatctcaactgaacccatagctcacagatttgcctggtctccctatccacttggccagggatcctgttttccccttgttgcccaggggttacaggcaagggagtcctcctggtcagtatttgcatgggctcttaagaaccccaaattccagacctcatgtttatgctctacctgaggagccatcttctgtcctttattattttgctgagatactatctgctgtataacatgtgttttttgaccttgagtctcaacactgatcctaaaaactggatatgtcttctggtttagtctctgttgttccctgcaaatagatcatataaagtgcccccccccattttttccagacagggtttctctatgtagccctagctgtcctagaactcactctgtagagcaggctagactgggactcagagagctgcctgcctctgcctcctgagtgctgggataaaaggtatgtaccatctctgcctgtctaggcctgttatttttaaccagtttttaagaagggctagcaaagagactgaataaaacgagagatggtgtgagacccactaacttggtgaaattagttcattattaatagaactgcaaactaatttgtcatgtgttgcagtgacaagtctctgtgtctacctgttcactgaaaaagaggcttccatgattaaggctaagaataccatttgtctaaatatttagaaaaataaatatttagaaggtactttgaccttgtgacaatttttctaaataaaagttttcagttgtaccatctcccccaacctatgaccaacccagctgtgggttttgaccatgtttacattatccgacatggactccttcagaatggccctcaaattcagcaagttggttacctccatggcagtaatgccactactgcacatgctacctggcaggttggtcttacagttcatagagttaactgtgggtgatgcctcttctctcccataaacctgcatagaaccttctaaatcattgaaagttaattggcagggaagaagcttatagctcagttttagcaaccaaggtatgtggtgtcttcagcaacagctctgttctctcttctcgtctccactactggagagatggccagagctcgttttattttaaggacatttttgactaataaggtttcccagcccaggattgggattttcattccataacctacagctcctaagaataggtttctttttcagctacattcaaaagccattttcaaaattttgttagtttttttaagatttaatgatcatgcttttgtcatatgcacctcacccatcaactcttcccaggtctactcccaattccctaattgcctaactctgtgtcttttttttcacccatcaaggcaaatttgtgctgcccaaataatcttggtgtatagtcttctgctggagcaacgtcaacttaccaaggactataatcttagtgaaaacaatctcttcctttcctaacagctaacaattggtaataactccacaacttagggtaggattttgtgtcaagctctcatgaaactcttatttttttttattatatttttacttgggtcataacctcttcattttggttgatcctttcccttaagctctcatctcccctgtccttccacccttgcctgcttaagcctttccacccccagccttctctctacatttagactgccttcatttttactctcctccctccattaagaccttcctctccccatgtaagccacaatatactggtctcaaactcactctactggaagatcttgaactcctgattctcttgcctctacttctcaagtgcagggattacagtcatatgccatcataccaacctagtgccctacaaccaagtgccttacaattcctttcagaaaatccattggaataattgagactggacttcacattatcaagagcaataggcactattaattctagactgatgttcacacggtgttcctcaggcccaaactgtccaaacagtagaaactgtaattagtgtgtttccagaggagccagatgaatgcattaagaatatgccttctgacctccgtgattgctttcattatgcaggattatcaagaggaaattgctgttgcccaagagaacaaaatccagctccagcaaatgggagagaggcttgctaaagctagtcatgaaagcaaagccgctgagattcagtacaagctcggcaaagtgaacgacaggtggcagcatctcctggatctcattgcggccaggtaaatgacaccaggtgcaataggatgcctgcagtggggatgtcaattagtcctccttcatctcagctagtgcagttcctcctgctgtgacctctccccaaactataaaattagtttgttggtgctctgtaagtgtaattttgctactgttgtgatgtaaatatttactgttaaatgtaagtatgttttggaggtcatgacccacaggttgagaagctaaagggaatgcagcacctatctccctttctgagtgactgtactgcctggggtaacactgtgctcctgctgctcccatgaatggcactttcattaacttcaaaagaatttagggagagggaaagnnnnnnnnnngggttttcatttgggggctttgtgggtatcccaacatctatggaggaaaaaagaaaaagccactccatcaatatttgtaggtgttcttatctggggggcagggggaggcggcaaaagagctaccacatccctgttatgtgtgtagttagttgggtgtgggcgtgagactgacctttgtcattctacttattcataaaaataaacagcttcattattgtcaactttctgctttgccataacagtgaccataattagtggtcttgtgttggagaggcagattatattccatttattctgtagacaggaagtgtgaataaaagggatgacaaacagaggaaaaacatatgagggcctttgccatcatttcaaatgctggtatgacttgaagatgcacaaggatattttatattaaaagagtaactgaccatggaagggcttcattttaagtgtaccttccttcatgttgggatgtcaatgccaagagacagctttgtccattgactcattgcatatcaaaagtctgagaataggggctggagagatggctcaaaggttaagagcactgcctgctcttccagagatcctgagttcaattcccagcaaccacatagtggctcacagccatctgtaatgagatctggtgacctctctggcctgcaggtatacatgcaggcagaacactgtatacataataaatacctaaataagtctttaaacaaaaacaaaagtctgagaatagtagctggtgctggggtgtgactcaaagggagaagggttgagtagcatgtgcaaggccctttgtctataaagtaatttgagtgtcacaaagactggaaggctgagaatgaatgccaccatagtgggcctccttgctggagtatatggtggcagtgcagacatggaaaaaaattgagcgaaaccattgagctccctgctcagggacatgcagggaaaggaatacatctttactgaaattaccctacagctgaaatgcacaatggttctgaatcccaatgtgatgtttagcctcacatctcagccaccaagatcataacaaagtcttattccagaagcagaaattgaaacctcgtgtgctataaattcccttcttggagagacctccccctgggtcaataccgtggggatttttgtgtgtgtgtcagatcctgactcatggaccaatgtgcttgtccgtataactccatcaaattggttaaatttctctcatgaatcccagggccacagtgatatggaaagggaagactcaccatgccaaaaaatatctcaaataggctttaactcagaacagttgtaggcagctggcttagtttctgctcagctgtcagctaacaatacatggagcacaatactatctcttcaaagtcatgcttatttacaacacatctgtgtgacgttttttcaggtgagaattttctagatattgttctcttttttaccatccccaaagatatacaaacaaacttgagtcagcagtatgttgataagaaatgggtggttttcaccatagtatctaagacagaaatgggtggttttcactgtagtatctaagacgttcatctatgaccacattttagaatgtcatcatgcagataaattcctgtggggaactttggtatagctatagtgttcatttctaggtaccacctataaagttagagcagattaaaggctgatcgtcagcttgctctggagtctgaagccacactggattctgtctgcctttcagcttctcccagaagacacttggctatcacatttgctttctgtttccttgttactgtgtgcaggcggggtgtacttcctccacacctgtctttagctatgaactggcagctgcttattcagtctcattcatgcctctccctctctccagcaaaaacagtgactcatgacacagaacagaacctggcacatcacatacttttggagttcttcaaaaattttaaattatatttatattaatatatatatatatatatatatatatatatatatatatatattttacacagctttcttcttccaagaatggaattcagatcatcaaaggcttggtagttgcctttacctgctaagccatctcactgtacccttcccctcttttct

SEQ ID NO: 12 - DNA, 199 bp, Cricetulus griseus
  gene 1..199: note = SYNE1
  source 1..199: mol_type = genomic DNA
atgaaactcttatttttttttattatatttttacttgggtcataacctcttcattttggttgatcctttcccttaagctctcatctcccctgtccttccacccttgcctgcttaagcctttccacccccagccttctctctacatttagactgccttcatttttactctcctccctccattaagaccttcctctcccca

SEQ ID NO: 13 - DNA, 6200 bp, Cricetulus griseus
  gene 1..6200: note = Smarcc1
  source 1..6200: mol_type = genomic DNA
gacatggaccttgtttgttttgatgtgcagaatccttataaatctcatttaatttgtatcttctatcagaaatgctttttcttttcactaatttcaggacatatataaatagcaggatgccaagaaactttcctactcaatgtcacaggggtcttagaggcagaagaaccaggttttacattcttgattctgataatattagaaaggagattagtatgaaagtgaaaatacataattactacatcctacacagagtgatctctttgtcccctgtaattgagcagaaagaccctggactttcctatgtgtggcactgactttcagtggtaatttctgcatgaggaggtgagtcaaatatactatttcccaatatattacacaggttgttgtttgtgagtatttcctgtatagttacatacaaaaataagcagaattgttgtggagtaataaaatgtacaatgtttgtggtaaatagctccctgaagaacactgtgctacacctattttgtaaatcaatagtttcctactttaagtgcatttctcagtgatatcaagaaactgctgtgtgatgggctctcaccacctgtttcagaagcaaccatggaggggattttaagatacattctgaagtctatacctgtggttcaattctcagaatgtaattttaattacttttctaaaatcctgtgagaactgcatgcatatatacaatgaattttgatcatttgtattcctactctgccctccaactactcctagaccatctcctaccacctccataatcatgacatctagtgcatgtacataagcctgcacactgaagcatagaaaaatctaccagtgccacagctctcaagaaacttgactctttgtaccccaacaggtgttagctgtcaaacaggtcctcagatatgtgtagggcctccataatccactgggattttaattggctttatcttgtgttggttttgtaaaggtgatcacagttgctcagattttataagttcaagggccctttggtgtgcaaaagataccattttgcagcagctcttcctaacctctgctatattttgaaggaagaagccactgcaaagagaatcagtgataaccccctaccaatgtcagtaactaaccatgaattaaagtaacaaaggacaagtagcatcagcaaatcagatcagcttcagccaatccctaagtatcacatttatgtccttgcccttctggaaatttctgagaagtaatcaaaaagtatgtaacccaaataggacagcatttcttccacccttgtcccagacctttgtccttcctaattttatttggaatgagttaaatattaaagattacatccccagagcacacatcctttacaggaacccatcaatgacattctgtaaagtgagacaagactaatatttaaacatttcttcacaccaaacattatttacacatacctaattaagaagttacagcatttcacatccttccaaaatcccttagcttagtagacaaataatacctaagtccattattaacacacgatttttagaaaatctttacccttatcaaatgataaattaggatctaaaatcatcctaatttatagaaacaagtcagcatttgctatgattgtgttagtgacaccatgtgaaaaaaatatgctagaaagtttaaatagatcgagaatgctccaaattcagtaaatgtacagctgcttcaaatccatggtttaattttatcttcttcacccttttagcattgaatcctgggactcttcagttcagacacctttgcaggtgctccacaaaagtaacctttcaatcagattaactgccagactgtgacatttgatgtgtcataatataaggctttgtgaattttaaatggttcagcacatgaagctgagatacagaaaagagtttgtaaggtataatttaaagactaattagtaaaaaaaatgtattatatacaattaaatgatgtaattatgaaatagttgatttgccagacatggtagcacaagtttatgatcttaccacacaggagaattaggcagaaggaacaagcatgtaagactagcttctattacacaagatttgtctcgaatatgatgaacttcgactatgccattatgactgtgtacctactgagaaaaagaattgcacaaacttcttaattctatgggaaatggaacaatgattataatataattttcaaacctgtttggaaatatttggaaatgtaacttcctatatgccatttgtatattaattgtattctagttaataatctgtttttttgaagtagttatgggccagtaagcttaactacctgaataaagaacttgaacaggaagtccttctcttttgttcttttgacttcttcaatattggaacaaatgttccccagttttcctgacacagagactcttgcatgtggatcatggtgtagtaaatgcaaagtggtcttggatgtctgaatttgcttggatgatttgtataacattgtcacactctatatacggatcccagcaagtggggatagtgctacaaagccttcctaacattgacctcaattcatgaatgcaatgagggcaaaaggtaagagtcaatacaaaactccgtcaagggagttttacaccctttagaaaccatataaaggaaaaagagagccaattccatcaaagctgtcttctgacttccccacaacacatatcatggcatgcacttttcttgctttccccatcatacacattccactaataaataagttaaaatgtaaaggatggtgattttccaaggtcagaaaaataatcactggaatatcagaatgatcatttgttgaaaatctgtagtaataatacctcaaacagaagcaaaccaacatctgcagttgcttctcttaatagtaaaagtatgtaatgttattttgcagtagaagacaaaatataattttgtgctataatttgttggtacttcatgagagctcagaaataggacctaaaaaagaccaaatggaaaggtaggtggacataagaaagcttatgcagagttcttcaaggagagccaagctgtgtgtttacattgtgttattctatttcttggaggtttagcagtgaaataacaacatgagacaagaaaaatagctttttatcagtaatgatagattgtttgaagagttatactgtaatatgtacatagagatcatggtatttaattctcaatttagcatgaacaaattaagtccatttttaaaaaagaggtaatggaggtacagaatgatcacaaattctgaggaggtttaggaaactttgtaaggctatgaagctattgacatgatttaaagactcctcatggatttagaatgtaattttctcagactcatggatatttgttgcagtcattctacactgagcagggttggtggtgacatcaggaacacacagaatttcagacctgcagaagacgcacggcatgttgtgtctgtcttggtactagtggtaacctccagtatccactctccagaaccaatatattattgagttgagttaagcatccactttcatatttggaatagaaactcattcttcctcccactaagacaaattccttaaaagtaacattatctttcatgttcaactttttatttaaaattcttcacattgactctggtctcaaaaggtacatacatttttaacataagaaaaataaatattagattttctcctttgcaaaattgccaaaggctattagaaaaaaagagagaaaataggcatcaataaataatacacaaaataatagaaactgaaaatgttagaaatatgaatagatgtttatttcttggtaatatgttcagactgggcactttgtaatatctagtgaacctactctgtctaataggacagattgtgaagtcagacaatctggatatatttaaattttaactctacctctaactaatatttcatgttggaaaaatttcaaaataactacgtaacagttttctcatatataatggaactattgggccatttctgtggcctcatgagcatacaaaaatgatacctttttagttaattatttgtcataattattgaaaaataatttaagtatgtactttccaaaccaacactatattctctaaaggagattcctatattaggttcagcacaaaaaaaatcttgagccaaaccctaatactatgtaacattgtaccctgtatgagccattccctttgatgatgaatgtaaatttttatgaattattggtttcattacaggttaaagaattttaatatgaattggtagctgatttccaaagtaggtatacaaaaccaaaaggagaataaatgattgataatgaaaatctagttacttgggattttaccaaaagaaatacttgaaaagaaaataaagctaaattaatgacagagacaagtactgtcctatattgtatttgattatatgtttgtggagacatctgttgttaattattttatattattcttaagtttagtggaagtcatagctgtagttaactccttatctccccacagctatagatctccaataacacccatctattttatctgtaagcagtatgttgaggagagagccttctagctttagaagtaacatttttaactgaaaataaattcttctctcatattgtatatcctgaccacattttcccgccctctatacctcccagcatccctaatctcttcttttccactttccctctgtttcctttcataaaagagtaaacctccaagagccaacaatcagacataacaaaacaagatacagtaagacaaagaaaaagcccttatatcaaggttggacaaggcaacccaacaggaggaaacacattctaacagcagcacataaaagagtgagagacacacctgatcccactgttaggagtcccacaaaaccaccaagctaataacaataatgcatatgcagagaacctggggtagctgcttgcagaaactgtgcttgcctctctggtctctgtgagcccatatgagccttacttatttgattcagtgagtcatggcctctgggtttcctccattctctctgacactgacaatcttccctccagtttgacttttcaaaagaaagtttggcaaccagctcagtgtttcaaataatttttaaatctattagcccatttgcatgagaattgattgtagaagtttatgcttctctgaaggctgtgatttatttgagcagttaatacttggtacatgattatttaatatgttatatgtgtcttcttttgtcttataaaatatatgtcctgctttactttttacctggtcaactgataattacatagattatcagatgcaacaaaagtttttgtatccatcagaaattccccaaaatgaatgcatgtagacttcataaggaagccttgcttcatttcaaagcactttctgattcaaaccaataaaaaccaaacaaaaaccctttaataattgtgttcttttactaactagcatgaagattaaacttaaaaaaggatactcaaaatcagatgcaatatttcttcaataatatttttaatcacggttcaggtaagaaaaaaattgaagattgaaaattaggattagtgataaagacaatgactagagaaaagaggaaagtgattaaattagaaactgtgaatgacagtagctttgattgtgattgacagagaacaaacgagtgtgaaactgctcatctcagttactaagcgcattcaccatttttcaaaactacagtaaagataaaccagacagaaaacaaaactgagctttgtagaaaacaaagattaatacaaaacaactaataataaaaaatagcataaatggttatggtaggcgagcaatacacatttccagtgagtggtataagtcttcttactgtcaatatagaatcagatgcaatcattttccttgctgcaaagatgattctttatggagccctttaaaatatatgcatattggtcagttttatgtcaactttacacagacagcttcatttgagacaaaggactcttaatagaggaaatccttccttaagattagacgataggcaaatctgttcagcattttctggtttaatgattcacatgggagggtctgaccccatatgagtagtgacagctgggcgtgtggccctacttgtataagaaagcaggtcaagcaag

SEQ ID NO: 14 - DNA, 199 bp, Cricetulus griseus
  gene 1..199: note = Smarcc1
  source 1..199: mol_type = genomic DNA
taaaaaagaccaaatggaaaggtaggtggacataagaaagcttatgcagagttcttcaaggagagccaagctgtgtgtttacattgtgttattctatttcttggaggtttagcagtgaaataacaacatgagacaagaaaaatagctttttatcagtaatgatagattgtttgaagagttatactgtaatatgtacata

SEQ ID NO: 15 - DNA, 6200 bp, Cricetulus griseus
  gene 1..6200: note = RSG19
  source 1..6200: mol_type = genomic DNA
caggacctatatgttggctctcaaccatttgtaactccagttccaacaccttctggcctctccaggtatgcatgtggcacacatattcaggcaaaacattcatacacacaaagtttaagagccatataaagccccttagaggatgtgggcactactaccagccaacagggctctcagcaatctctggacagggtgatgctgtggcagaggcacctgtctacaagtagtttcttcttagcctgtggagggtctagggaacaggactgggtctgagtcctaaaatccaccccatcccacccctatatgcctcagtgcttctgtatctcttctatgagctgctccccaggcccatataccatgtacccccaggcctatatactctggttttgccctctttgagccatgtacccctgcccaaatgccctggggtcttcttcccagtataagctgcacccttaaggtccacataccaggagcagctgcagcagcagcaccagcataagcagcaggggttgcgactggggggtcctgagggggctgcatcatggctggacatcgaggggggcctgtccgcctcctctggtcctgtgtgctgaggaagagggggctgcctcaacctccattccagaattcactggaccctatgtctgcccatctgcccaactggctgtgcccccaagggcctcaggtgtccaggaacccaattagagggaggaagtgcctacctgtttctccgcctcatgtggggtgggcatgtgtgggtggagagggttgcacagattctgtggtgccagctctggaccttcactgcagtctgggagcttggatctgagaagagtgttgggagttctgactgagggcctgtgacctgggcccaccttgtaacctctgcaaccacctcaggtccctcagagggagcttgctcagagctctaccccaagtctgtgtgctaaccccatatggaagtgccccaggcaatgatggggctactgcagttgggcctcccacaaagggctctaagatacccccatctactcagtccccaagaagccggaagcctgggttcctctttcttggcttccggctcctggcccctcctaaggggactggagctacaggctggtatggagatggtaggatactctgatggctccctccctctaggtaggtgggtagacatgctacccagatgactgcagagggctaggtctgaggcaccagagtacttgagtagaattcagaacaagacttcctgaaagtgaggaatggaggtggggggttactcgagagatgtgtacttaggtaacaaggctcttaggtccttggctgcgtcagacacccccacttcaccctggtttccctttttctcctgaggatgcagaagcagggagtgctagccatggaagctggggtggcaatgtgggaggatcagctgcttagctggagccttgggctcttcaatgggttttcatatgatttatcattcttgatgtttggaccacaccttcacagggggttctaggaacctctcaggcctctgaaagctgacttcaaattccagtgtccccaggaaaaacagaagcaaagcatccaattagcaccctggcagcagttttgaatgcctcctctctccccagcctgtgcccatttctgaccaggtggaggctaggctatccaggccttaagatctctgctctgcccaccttcctcacattaacctggggctcacgttactttgtcgatgaaatccaccctcctgtagccctgaatccagcagagggaggccctttatcctcttctgcctgaggtctgtacactgagggcagccccaccacctggctcgatttctgagatggtgggttcccaagtctcccagcgtgcaaaccaggacacaaaagtagcttgggctgtacttccctggggtggagcttctagggaaaggaaggggtgtagtagcctaaggtctctaggctctccagagtcatcaccctgcagaccatccctcagatgctccatctccaaccagctgactggacagggaacagcctggggtgtgtggggcctggatgctggggtccagtttgtgcagacgcaggtgtctgccattttccccagctgcaggctcttgtcctggctccttgcacccatcaaaggtcggttgggaccacccatgtcgtccagagtgctcttgactaccgcctcccttctttctagggaaggggagcccagcatctgaattagggttttcctgccccatctccggatactggatggctcattccctccccaagcctcccaggcgttggcctcccaagtctatgctgagaccaaatgcagcaaatctggtctctggggacagaagctccctggggaatggctgccgtgttgctccacagaagaaaatgttcaagcccgaccagtccaaaaaaaaaaaaagaacctttgggggggggtaacaggggttccattcccacttccatcccacactgtcattgtcctacctgtacctccatggcgggccagacctctctcaccatggcgaaccccgctgcccaagcccacctgtgggatggtaggcccccacccagttactgctttctgctggtggggtcgtctggagggctggtctcttcttcgcggtccctctcgcagtctctgacgcccccacccctttcttaaggaattcgccatgaggccccactcaccagcgacctaaaggcggatgggggcgggagggccaggttcggtctgggccccaccctggctgccgaaggggcgtgctctaaagcagcagggacttaagtcagacagcaagatgtactcctgggtattcgcgagataggaaggcgcacagaatccctctcgggtggggctgtggagggggcgcaacattcacccctaaggctcgccgggccgagtggctagtggacccaactcgaagggtgggtaaggtggtggatcggtgtctggcctggcccctccccactaggctagcgggcgggagacacggaaacctgggttcttccggcccccacctttagcaattacttctcaaagctctgagctgaagaaaaaggggaaccttgctgcggctctccctcccccacgcgcagggggtgggctccggtcccaccgcgacccaggtccacgtgggctggtcgctgaagtccgggaacagagccggcatctacatctccggggcccgcccgcggtccagcgccgcactcaccgcagagtccccgagtcacagcgcccgcgcgatccgaagtcctgcttgtcgccggggagggggcgcaggcgcagtgcgcaggcgcctccacggtacttccccaaagagaggggccgggacttcctcgagccccagcgcctgctcgcccgcagtgccccgccccgcgcccgctcccgcgccccacccgcgctggcgtgtcgtcctgcggtagcgtggcatggtgaccctgaggggtgagtcgtacacagacagtggattgagccggcgctccgtctggttagctaggttttcccagcctttcctttctgtggtagtgcagtgtggggcaccagagctgagcccagtgtgcttcttggcaggatgagaagaggcctttgggaaggactggcctgttgtactgccctgtccgccccaccccttcgcatttctgagtctggtctgtcactctgctgtccacagagaaagggagattcaggaactgcagcttggtgggcactgtgaatgcaggttcttatatcaaattaccccgaaagtttctggggcctagttgagtccctccctattgacccctcaaattgctccaagatagccttttctgcaaatggccttactctttggccagctcttcagatcctttattattgggtgcagatttgaattagctcattatcccagcatgctctgggcaagtgtccaggggccctgaccctactttagacttggtttgtagggtgtgtgtggttgcttgggccatgcggttcctgcccttcttagcactggaacacagcctaaccagttcaggtgctagggtcttggaagaaaaaaaaaaaaaaaaaaaaaaaatttaaaaaaactttttaatcgcacaggttgtatatgctgaccacagaagttagaggtgcaaagcaaatacccactcttgaggcagcgggtcccaggcagacagactgacctggagctaactgcagtggactagaatgggagacaggcccaaaagggatggggtgagaggtgaggagggcaggatgttgccatgatgttcagggagtctggatgaagagagaacattggttgagagcctgaggctaccaggctttctctaatgctgtgtggggcttgatgaaaaaagccagaaccctttagctgccacctgatggattccaaagcaaggtagaggctaagaagcccatctaaacagtagtagttgctttagataatagtcctgagaagtggacacagtttagaataaggaggcccagtagaaatgggtcaataccaggtggagacaacaaaacaaagctgattctgcagtatttggtgtgggcaactggctgtgggtagaagtcagtatgcgttcttcccctcagttcattttacatgcctacccacttgttctctgctaccttacatctgttctatactcaattagcatctttaagcacagagaatgcccctaaatctaggcaggagaccaggagcactgagcaagtgacactagtgaggatggaactttaacacaatttacccttttctagagcaggacccctactcccagccccacccccccaccccggcaccagccactcataagccccacttaactgtgcatgggccacaggctttgtatcctcgttggattttcttcagacagagggatcctgtgccaccttccttagcctactctgtaaacccaatccctcactgatgtggagatcaagtggcactcttaagctggtctgacacttggtgtagagctcttttgccattgttatgctggccttctcaggatgttggtgtgtgtgtcctcagccctctgctctgaggtacttatctgaattactcactatgtgggacactgcggtaatcttagacatctctgtgatcaccatgaagaaatgcagggttggaaaagtgactttactaaatagatgaagtttttctaggctcttggcaaatccttggcaagctcctctacaaggagcttgaccagaggagcccagcattggctatcatctggtgtaattgactgtcattagaagactacaatctgggtgtgtgtgaccatcattcctggatgaagagactgtctccttttccctgtctacacccatgtccaaacctaccatttccctgctctgccatcctccccattgcctgaaaccccctcccctcctcctaagagctgctgctgatttgtgagtgctcccatctgggtttggatcaaggcccagggcagcaacaggccagaaagtgagaagggtcatgcgcagggggagaagaccagctgaggaaacagagccctgggaactggccatcagtgagtaagagctttctggaccacagttttgatctcttcttcctttctgttctctgttccatgaagagccagggggagctcccatgcagggacagggagctgtgtacctccccatagtttctgcctctgtccagcctgctgggtagggactaagaagaaggacaaggccaaaggactgaagggcaagagaccacaggttctgcaaagaacccatgctgtggagaagaggaagaagagcctcccagaaaccgggggcttttcagagtctagtggtcagaacgggatgagtggcttacttcctgtgctccatatttggtggatgagtgagcacaggaggctgtttctgatgaaagggaggctgtgggtgagtcttctgtcccaccatccagggaccttggtgaggagcaccctgttcacaacctggtggtcctctgggcatgactggactctccaaaggtgagcttattccctctcccagaatgccaccccagtcttcagatggaatgatcctaatttaggagacagccctgatttttgtgggtgctggtgtctaggcaggctcattcatccctattcttttccacactagttcacgccctccccgcatctgtggctttgaagggcacccattacctgatgggggcaggtggtttg

SEQ ID NO: 16 - DNA, 199 bp, Cricetulus griseus
  gene 1..199: note = RSG19
  source 1..199: mol_type = genomic DNA
ggagacacggaaacctgggttcttccggcccccacctttagcaattacttctcaaagctctgagctgaagaaaaaggggaaccttgctgcggctctccctcccccacgcgcagggggtgggctccggtcccaccgcgacccaggtccacgtgggctggtcgctgaagtccgggaacagagccggcatctacatctccgg

SEQ ID NO: 17 - DNA, 4537 bp, Cricetulus griseus
  gene 1..4537: note = Tenm3-fragment
  source 1..4537: mol_type = genomic DNA
cttccaagtaaatatccacaactacacggttcatgagattactcgcaggatttaggattttaaagaataatagtaaacagaagcaaggaagtgatcgggtttgaggaggtcacacctctttaatgcacttaaagaggacaggaatacagtcccagctgaagtccaagagaagacagacaaagggaagggcgcacttaatacagaggaataaatactgaagggagctcgggctgaaatggagctagaactgaaaaattcaatatcccatctgttagggtcacccgaggacaggacaccagacaccttcaggcaaacagcttttatatgtgagaggagtcatggagagaaccagaccagagcctagccagacagagacctgttccgtaccatagtctaacggctgctttaaacacagtgtgggcttaaatgtctttcatgtcaggaagggaggacggcttgggagcattgccaggccacacataacactttggtggagactaaacaggatggtggtctctttgtccttctttcaaggcctcctggaagatttactaaggaaaggggattactggggagatgtatcaaggtttttatacacgcaagggcattgctcggccctgtggctgcatctggttttcattgccctggctctcaagggagtctccctcacatagggtcaagcaggagataggatgtcaggaccgggagacacagcagagaaactggagaacaatatctttaaatcaaagaaagaaaaaatatttaaaaggaatatgcaagaatttggggacaccatgaggcccaaacttatgagttacccgagaagactctcaggtggaagaaaatgaatggggtatccagagaagacccatggttgcaatgcttgtcttagttgtgaaccacactccagcagtccacaatctcttgaccaactctcaaatgccatcatctgttgaatattcccaggaattggtccatgagttccctgaaatccctcaagatctgataatgctcaccagacccgtcctcacagacactcacgagatatgctccactaatttcccaggtatttcctaatcttagcacgttgacaatcaaggctgagcatcccaacagcataaagttgaccaaggagcacgggaaaagttgcacagcatcgctactcatcctgaggattaaagtgaaaacaccacgaggaaagattcctggtttgtcgctttgcttgaacgagcctggaagtttgcagctcatcctcacacagacaccctggtgaaccaactagaaacctagcagttctcctaggctgtgcaagaaaggtgagcacacacaggaggaaatacataaagagactggagttcagcgttgaagtcagtaggtcacaggcaccctgggtccttgtcacacttgcctgaccctgaccccgccggcacaagagggtctggttctgcggttcctttactcgcagcaattgagtctggttcccaagaagacgccccacgcaggacgaggagagcgagcgggttggaaggaatccacggccggaggtgcgggagtgtttcccggggtgaccagcagggggcgcggggcgggaaaggccttcggggctcctgaagttggggttcccgggaatgaggggagtgtgtgagccgggcgggctgagagcaggttagagccaggccgagagcggttggggagaaggcgaactgggcgtggtagttttcactctacactccgcccacagtgttgggagggcgagtacgtcatcgtaactcagcgctaactaacggtttgatgtgagctgcttccgccggctctggtggcgcaggccggaaggatttgctgaaggaggcagaggcagggggatctggagttcgaggccagccaggactacacatttttttttcttgtcctccaacaaaacatccacagctacaggctacagtaaaattcctacacccacaaaggctctccacactctactctcaacctcatttcgctcgcgactgacacccaaccgacaccatcttttctagacgcacaggcgcctgctccaccctgctgctcacaagcctttgctcacacaccgactcacacgctccacctccgcgctggccaatgctcgcatagtctaacggctacttgaaacccatagtgtggacttaaatgtcttttacgtcaggaagggtggacggcttgggagcattgccaggccacacataacactttggtggagactaaacaggatggtggtctctttgtccttctttcaaggcctcctggaagacttactaagcaaagcggggattgctggggagatgtatcaaggtttctatacacgcaagggcattgctcggccctgtggctgcatctggttttcattgccctggctctcaagggagtctccctctcattgagaagactcagtggaaagccttcctagttgacatagggtcaagtaaagacagaatgtcaggacctgcagacacagcagagcaactgggaaacaataccttaaaaacaaacaaagaaaaatatttaaaaggaatatgcaagaatttggggacactcatgaggcccaaatttatgagttacctgagaagactgtggggtggaagaaaatgaatgcggtatccagagaagacccatggttgcaaagcttgaccagctctcaaatgccatcatctgttgaatattcccaggaattggtccatgcgttccctgaaaaccctcaagatctgataatgctcaccagacccgtcctcacagacactcacgagatatgctccactaatttcccaggtatttcctaatcttagcacgttgacaatcaaggctgagcatcccaacagcacaaagttgaccaaggagcacgggaaaagttgcacagcatcgctactcatcatgaggattaaagtgaaaacaccacgaggaaagactcctggtttctagttttgcatgaaggagcctggaagtttgcagctcatcctcacacagacaccctggtgaacctactagaaacctgacagttctcataggctgtgcaagaaaggtgagcacacacaggaggaaatacatagagagactggagttcagcgttgaattgtcctccaacaaaacatccacagctacacactacactaaaattcctacacccacaaaggctctccgcactctactttcaacctcgtttcgctcgcgaccgacacccaaccgacaccatcttcttcagacataatgactgtcagtgtacaaattaaatgaattatttactaggagctgaaagaccattgcaactgctcgccaattcgactatttgagctgaagccggagttgtctgctccacatatttctttccatcaataatataggcggctctcccattggaggagccatcagtaaaaactaacatagcattttttacaggattgcttttaacaatttttggaaatataaaaggatgcattagtgtaaattgcaacagtccatgagctggaaactgaatatcaattctccctaaaaactgatcaaaagcaatcgcccatgaatcactgttttggaacaacccattaacctgatgcttggtgtaagggacatgtattatatttggctctttgccaaaatacttcctagcttttacaaggcatttttgtaccatgcaggctactgcttcaaaataagggtctaatactttggatggcgagactggtaggtgtagccagagtaatggtccctcctgccacagaacagaagtcggactatgccttgtggggagtatataagcctcccatggctttgcatagtcaatataacatatttgttgacgctgaatcgcctcctccaattgtagcaggactcgtctaccttcctctgttagctttctaggtgaatttggatcattatctccctttaaaatatcacagagcggtttcaaatcaccagtaggctctctttaaaaaggacgtaaccattgaatattccctattaatttttgaaagtcatttaaggaccgtaagctatcttttttaatctctaatttctgaggtctaatctctttagcatataacatatgacccaaatattgaaaaggtggctgtctctgtaccttctctggagcactcactaagcctgctctcttgagactttgctgtagctgtccataaatctcgagcagaaccgcttcatatttatggacaagtaaaatatcatctatataatgaacaataaagacttgtggaaatctgtccctaaccatttgtatagctcgagacacaaacttttggcataaagttgcactattggccatgccctggggtaaaaccttccaatggtacctcctcatggctctttaaaattaactgaaggaatgctaaatgcaaacctatgacagtcctgaggaaccaggggaatagtataaaaacaatcttttaggtctacaacaatcttataagtaccctttggtacagctgcaggaatgggtaatcctggctgtagtgctcccattggctgcatggttttattaactttcctcaaatcttgt

SEQ ID NO: 18 - DNA, 4109 bp, Cricetulus griseus
  gene 1..4109: note = SIVA1-fragment
  source 1..4109: mol_type = genomic DNA
ctgaggaccaagcaggaggaaaatcacaataacattcttgaataaaacaaccctattcctaaccctttggaaagctgccagtttgcttagaagataagcacatgtccccctctccctctaacacattcacgttcggagggaagagggagccccattcccgagtagcacccaacactgaatgatcaatatgtcagaaaaggcctggtccaaggttgtccataggaactaaatgcatcatagccaaagcttgccaatggccctggtgcctaacaggcagatacacaactttaggctttctagacagaagaacacccagtatcaaaacgaaccagctgccacagacttgaactagagggagcaagctcagaactacgggagagcagccagatacatcggcacacacagaatgagtactccctgtatgagattctgatgccatttggtgggaactttggaaaaagagtaagaaaaagctcagtgtcagacattttacaagcatactctggctgtggcccccaactgaagggaaaagacagaagaaactatgacatgattacccctctctaacacccaccggcagccagacccagtgaaaccctttggaagcttgcagggaattgtgggaattcttggccgggtgagggggtgggggtgtcattatcttaatgtgaacagcagtcctggtggtggttccctagccatgttcccgccccgtctgtcccactggatttaagccttacagtaggagacaagcccatgcctccacatagaggtggagcctgttccttacagttctacaacaggggacaccacccacggggaaggaaacacagaaggcagttgtcacttctacaggtgtttgtcatcagggctttaacctgtacacctacttggcacttgtcctatgctattcatgttgaagtcctaactcctaagacttcagaatgtgactatctggatacagccttttgtttattttatttttggtgttttgagacagggtcgcaccacacagcttgggctggcctcaaactcacagagatccgcctgcctctgcctccggagagctgggattaaaggcgtgcgccgccaccacacctggctcctgggtatatatatattcttaacgagttaaaacggggtccttagggtggacccgaactcaaagaggttggtgtttttatgagatgaggactcagacaccccatgtagtttccatctgcagatcaaggaagatgagaggcctgcagagaacccaacgccttaatctgaggctgtgcctttgtaattacagatcccctaattggccttctccctttccgaactcgggaacgcaaactcaagtactgggactgggggtgagggggtgtgtgtctcaaaatctggagaatgctgagcatgcgccaggcctccctcgcaccgtgatgagcgcaaaactcaatgcacctcaacaagtcgcccttaggttcagatagagtgtggaaagaatacaggactcaggaggccctcggcaccgctgctgtgccgactgtgtgcaccgcgttaggagccgcccaggcaggcagtgccagcggtaaacgctcacccaagctcgggctcacggacgcaggaggaccgcagggagagatgggtgccggcacccaccctgctgctgcgactcgtcccccgggaagaccacccatcacagttgctaagcgaccgcggagactttgtgccgcgcaggcttacacagagccccggcgcgtaagccccgcccctgggtagcctcccgctggtttcccgcgccacaccctccagagcccccgcctcttaatcctcggcctatcccgagtcgtctcgcgcactacccccgcccacctccaactctcggcctatcccgcgccgcgccacgcgaagaccccgccctccttgccatccctttggcctttcccgcgccccctgagttccacccacttcctccctcagcctattgcgcgcccttgagccccgcccccggcctctccccggcctatcgggctccgcgccgtcgccagccccgcccccgccggcgttgtgagcgcgctgtgacgtccgcgccgctgtggtcagtgtttggtacccgctgccatgccgaagcggagctgcccgttcggggacgcttccccgctgcagctcaaggtccatgtgggcccgagagagctgagccgcggggtgttcgcccagcgctactcgcgggaggtcttcggtgagtgcggagttccgtggtagggcgcgcagcgccgcgccgtgggagaccccaactggcttgcgcgtcgccatccccggggggggaggcggcgtggggggggtccccggggagcggctccgggggaaatgcgagtgtagccgaggactgtcgagcgggagtcggccccctcaagtgggctttctggcggcagggtgttgctttgcagtgatggctctctggggccgatgcaacgcggcttacctggcttagggcgaagtttatgcctgtagttttgagtggtgcgctgtgcctttgggatgtgtcgttaaagcccaggctgcggaattacagactccctaatgcgccgtgtgtgtgtgtgtgtgtgtgtgtgtgtgtgtgtgtgtgtgtagctgatgggccctttccctttctgtactgtggaatgcaaactcgagtgctgagacctcaggggtgatgagtgaagtgtgaggcctgaacagcaaagcgtcatgcactcatttaaaagaaacaaaagtagacatgacgggagtcttggcattcgcccttgatgctagcaactcaccaggcagaagcaggcggatctctgagagttccggggccagcctggtctacagagcgagtgccaggacagcctccaaagccacagagaaaccctgtcttgaaccacccccaccccccaaaaaaaagaaaacctaagtataattggaacctagcagcctggctctactcttttaaagacttatatcctggagcacttgccagggccagtcagaaccagccaggtcagggaggggtgctggtttctggggtgttgtatagtcatacagtacacacaatttgaggcctgaaggatgaataccaagcctcggcctacactctggactcttttgtgggccaggagtccttgaggagaaagattactctcaacatgggaatcttcctatctccctctttttcaagcaggcttttacaatgtatcttaggctaaccttgaacttaaacactcctgctgcctcagcctcctgagtgctgggatgtgcctctgtatctactttctatcttaaagcaggaggtggcacagactgtaactggcctgataacagccactccctgtgactttttgctggctgttgctgctgccagtttcacagaggggcccctgggtctgacaggtctcccctggctgtatgtgggagtgagcatttctggaaccagcacacagtgtagcctaatgggaagcccctgttaaagcccacttagcgctgggatagggggtgggtggacctggaaggttctgggagacctttgtcaggaggttgctgtctttgtcccctatagtaagtgcagttgtccgctggcctgatggtgattgtaggcgctgttttgaacctgtgtgtttcctgcctctttggggcacttgctctggagagtgagtggttcaaggccagagctttctctggcgtgaaagacaggtgcttataggagggtgaagagtaagacactaacccagtgaagtaaggttagctgtggctgctgagataggctaatggaaggaaccctgcgcccagcacatcggggtggtggggttgggctgcagcatctgcaggctgctgtggaaggagcgaacagtggagacagaaaggacgggagcattttcagcttggaggcagggaggccctggcagtgtcaccacttagggaacaggcacagaggacgacgcctatgcaggggctttgcagttggcagtgttgtctttaggaaggatctttcttccccagaaagaaccaagcagctccttttccaaggggcccaggcctgtagagaccacatatggggtgaaagatgtcccatcatccacctgccggagtcactgaagcctggc